European Patent Application EP 4 656 649 A1, published December 3, 2025. Title: ANTI-ACNE RECOMBINANT PROTEIN VACCINE, PREPARATION METHOD THEREFOR AND APPLICATION THEREOF. Applicant: WestVac Biopharma Co., Ltd. Application CN. The sequence listing filed with the application follows.

SEQUENCE LISTING (4 sequences)

SEQ ID NO: 1 - protein, 240 aa, synthetic construct
MVEPTTTISATSTHELSASDARNSIQLLNAHIATLQSVQKSVPGSDYSDQIRDLLKAAFDLRGLIETLAHGGIPFYDPSTIMPRIKLVATTIDTIHTATTTLQNKVRPAHVELGLEVTKAVLLTANPASTAKELDAEGAALKARLEKVSQYPDLTPNDVATVYVRTNFSKTIWQVRANRDRYILGHKSAAVYKTLNHAITKAVGVRLNPKTTVGNIQAARTELLAAYQTAFNSPDVKKAA

SEQ ID NO: 2 - DNA, 723 bp, synthetic construct
  source 1..723: mol_type = other DNA
atggttgaaccgaccaccaccatcagcgcgaccagcacccacgaactgagcgcgagcgacgcgcgtaacagcatccagctgctgaacgcgcacatcgcgaccctgcagagcgttcagaaatccgttccgggcagcgattactccgaccagatccgtgacctgctgaaagcggcgttcgacctgcgtggtctgatcgaaaccctggcgcacggtggcatcccgttctacgacccgtccaccatcggcccgcgtatcaaactggtggcgaccaccatcgataccatccacaccgcgaccaccaccctgcagaacaaagtgcgtccggcgcacgtggaactgggtctggaagtgaccaaagcggtgctgctgaccgcgaacccggcgtccaccgcgaaagaactggacgcggaaggtgcggcgctgaaagcgcgcctggaaaaagttagccagtacccggatctgaccccgaacgatgttgcgaccgtttacgttcgtaccaacttctctaaaaccatctggcaggttcgtgctaaccgtgatcgttacatcctgggccacaaatctgcggcggtgtacaaaaccctgaaccacgcgatcaccaaagcggttggtgttcgcctgaacccgaaaaccaccgtgggtaacatccaggcggcgcgtaccgaactgctggcggcgtaccagaccgcgttcaactctccggatgttaaaaaagcggcgtaa

SEQ ID NO: 3 - protein, 240 aa, synthetic construct
MVEPTTTISATSTHELSASDARNSIQLLNAHIATLQSVQKSVPGSDYSDQIRDLLKAAFDLRGLIETLAHGGIPFYDPSTIGPRIKLVATTIDTIHTATTTLQNKVRPAHVELGLEVTKAVLLTANPASTAKELDAEGAALKARLEKVSQYPDLTPNDVATVYVRTNFSKTIWQVRANRDRYILGHKSAAVYKTLNHAITKAVGVRLNPKTTVGNIQAARTELLAAYQTAFNSPDVKKAA

SEQ ID NO: 4 - DNA, 723 bp, synthetic construct; identical to SEQ ID NO: 2
  source 1..723: mol_type = other DNA